European Patent Application EP 4 400 115 A2, published July 17, 2024. Title: ALUMINIUM COMPOUNDS FOR USE IN THERAPEUTICS AND VACCINES. Applicant: Valneva Austria GmbH. Application EP. The sequence listing filed with the application follows.

SEQUENCE LISTING (1 sequence)

SEQ ID NO: 1 - protein, 223 aa, synthetic construct
  REGION 1..223: note = OprF-OprI fusion protein from pseudomonas ae.
AHHHHHHAPAPEPVADVCSDSDNDGVCDNVDKCPDTPANVTVDANGCPAVAEVVRVQLDVKFDFDKSKVKENSYADIKNLADFMKQYPSTSTTVEGHTDSVGTDAYNQKLSERRANAVRDVLVNEYGVEGGRVNAVGYGESRPVADNATAEGRAINRRVESSHSKETEARLTATEDAAARAQARADEAYRKADEALGAAQKAQQTADEANERALRMLEKASRK